European Patent Application EP 4 349 989 A1, published April 10, 2024. Title: GLYCOSYLTRANSFERASE AND APPLICATION THEREOF. Applicant: ABIOCHEM BIOTECHNOLOGY CO., LTD. Application EP22815324.3. The sequence listing filed with the application follows.

SEQUENCE LISTING (112 sequences)

SEQ ID NO: 1 - DNA, 1371 bp, Artificial Sequence
  Enz.1
atgccgaacactaacccaactaccgtgcgtcgtcgtcgtgttattatgtttccggttccgttcccgggccacttaaacccgatgctgcaactggcgaacgtgctgtaccgtagaggttttgaaatcaccattctgcacaccaacttcaacgccccgaaaaccagcctttatccgcacttccagtttcgttttatcttggacaacgatccgcaaccggagtggttacgcaacctgccgacgactggtccgggcgtgggtgcaagaatcccggtaattaacaaacacggcgcggatgaattccgtaaggagctggaaatctgcatgcgggatactccgagtgacgaggaagttgcttgcgtgattaccgatgcgctgtggtacttcgcgcaaccggtggcggacagcctgaatctgaaacgtctggttctgcagaccgggagcctgtttaacttccactgcctggtgtgtctgccgaaatttctggagttgggctacctggatccggaaactaaacatcgtccggatgaaccggtggtaggtttcccgatgctgaaggttaaagatatccgtcgcgcgtattcgcacattcaagaatcgaaaccaattctgatgaagatggttgaagaaacccgtgccagcagcggtgtgatttggaacagcgctaaagagctggaggaaagcgagctggaaaccattcagcgtgaaattccggcgccgagcttcctgcttccgctgccgaagcattatagggcttcgagcactagcctgctggatactgatccgagcaccgcccaatggctggaccagcagccgccgagcagcgtgctgtacgttggctttggcagccagagctcgctggaccccgcagatttcctggagattgcgcgtggtctggttgcgagcaaacaaagctttctgtggctggttcgtccgggcttcgtgaagggttatgagtggattgagctgctgccggatggttttctgggtgaaaaaggtcgtatcgtgaagtctgctccgcaacaagaagtgctggcgcacaaggcgattggtgcgttctggacccacggcggttggaacggcaccatggaggccgtgtgcgaaggcgtgccgatgatctttagcgatttcggtctggatcagccgctgaacgcgcgttacatgagcgaggttctgcatgtgggcgtttatctggagaacggcttcatccgtggtgagatcattaatgcggttaggcgtgtgatggttgaccctgagggtgaggttatgcgccaaaacgcgcgtaaattgaaggataagttggatcgaagcattgctcccggtggcagcagctacgagagcctggaacgcctgcagagctatattagcagcctg

SEQ ID NO: 2 - protein, 457 aa, Artificial Sequence
  Enz.1
MPNTNPTTVRRRRVIMFPVPFPGHLNPMLQLANVLYRRGFEITILHTNFNAPKTSLYPHFQFRFILDNDPQPEWLRNLPTTGPGVGARIPVINKHGADEFRKELEICMRDTPSDEEVACVITDALWYFAQPVADSLNLKRLVLQTGSLFNFHCLVCLPKFLELGYLDPETKHRPDEPVVGFPMLKVKDIRRAYSHIQESKPILMKMVEETRASSGVIWNSAKELEESELETIQREIPAPSFLLPLPKHYRASSTSLLDTDPSTAQWLDQQPPSSVLYVGFGSQSSLDPADFLEIARGLVASKQSFLWLVRPGFVKGYEWIELLPDGFLGEKGRIVKSAPQQEVLAHKAIGAFWTHGGWNGTMEAVCEGVPMIFSDFGLDQPLNARYMSEVLHVGVYLENGFIRGEIINAVRRVMVDPEGEVMRQNARKLKDKLDRSIAPGGSSYESLERLQSYISSL

SEQ ID NO: 3 - DNA, 32 bp, Artificial Sequence
  GT010-L308A-F
gctttctgtgggcggttcgtccgggcttcgtg

SEQ ID NO: 4 - DNA, 30 bp, Artificial Sequence
  GT010-L308A-R
ggacgaaccgcccacagaaagctttgtttg

SEQ ID NO: 5 - DNA, 32 bp, Artificial Sequence
  GT010-L308D-F
gctttctgtgggatgttcgtccgggcttcgtg

SEQ ID NO: 6 - DNA, 30 bp, Artificial Sequence
  GT010-L308D-R
ggacgaacatcccacagaaagctttgtttg

SEQ ID NO: 7 - DNA, 32 bp, Artificial Sequence
  GT010-L308E-F
gctttctgtgggaggttcgtccgggcttcgtg

SEQ ID NO: 8 - DNA, 30 bp, Artificial Sequence
  GT010-L308E-R
ggacgaacctcccacagaaagctttgtttg

SEQ ID NO: 9 - DNA, 32 bp, Artificial Sequence
  GT010-L308G-F
gctttctgtggggtgttcgtccgggcttcgtg

SEQ ID NO: 10 - DNA, 30 bp, Artificial Sequence
  GT010-L308G-R
ggacgaacaccccacagaaagctttgtttg

SEQ ID NO: 11 - DNA, 32 bp, Artificial Sequence
  GT010-L308H-F
gctttctgtggcatgttcgtccgggcttcgtg

SEQ ID NO: 12 - DNA, 30 bp, Artificial Sequence; identical to SEQ ID NO: 6
  GT010-L308H-R

SEQ ID NO: 13 - DNA, 32 bp, Artificial Sequence
  GT010-L308I-F
gctttctgtggattgttcgtccgggcttcgtg

SEQ ID NO: 14 - DNA, 30 bp, Artificial Sequence
  GT010-L308I-R
ggacgaacaatccacagaaagctttgtttg

SEQ ID NO: 15 - DNA, 32 bp, Artificial Sequence
  GT010-L308K-F
gctttctgtggaaggttcgtccgggcttcgtg

SEQ ID NO: 16 - DNA, 30 bp, Artificial Sequence
  GT010-L308K-R
ggacgaaccttccacagaaagctttgtttg

SEQ ID NO: 17 - DNA, 32 bp, Artificial Sequence
  GT010-L308M-F
gctttctgtggatggttcgtccgggcttcgtg

SEQ ID NO: 18 - DNA, 30 bp, Artificial Sequence
  GT010-L308M-R
ggacgaaccatccacagaaagctttgtttg

SEQ ID NO: 19 - DNA, 32 bp, Artificial Sequence
  GT010-L308N-F
gctttctgtggaacgttcgtccgggcttcgtg

SEQ ID NO: 20 - DNA, 30 bp, Artificial Sequence
  GT010-L308N-R
ggacgaacgttccacagaaagctttgtttg

SEQ ID NO: 21 - DNA, 32 bp, Artificial Sequence
  GT010-L308P-F
gctttctgtggccggttcgtccgggcttcgtg

SEQ ID NO: 22 - DNA, 30 bp, Artificial Sequence
  GT010-L308P-R
ggacgaaccggccacagaaagctttgtttg

SEQ ID NO: 23 - DNA, 32 bp, Artificial Sequence
  GT010-L308S-F
gctttctgtggagcgttcgtccgggcttcgtg

SEQ ID NO: 24 - DNA, 30 bp, Artificial Sequence
  GT010-L308S-R
ggacgaacgctccacagaaagctttgtttg

SEQ ID NO: 25 - DNA, 32 bp, Artificial Sequence
  GT010-L308V-F
gctttctgtgggtggttcgtccgggcttcgtg

SEQ ID NO: 26 - DNA, 30 bp, Artificial Sequence
  GT010-L308V-R
ggacgaaccacccacagaaagctttgtttg

SEQ ID NO: 27 - DNA, 32 bp, Artificial Sequence
  GT010-L308W-F
gctttctgtggtgggttcgtccgggcttcgtg

SEQ ID NO: 28 - DNA, 30 bp, Artificial Sequence
  GT010-L308W-R
ggacgaacccaccacagaaagctttgtttg

SEQ ID NO: 29 - DNA, 19 bp, Artificial Sequence
  ET-F
cttgtctgctcccggcatc

SEQ ID NO: 30 - DNA, 20 bp, Artificial Sequence
  ET-R
cttgtctgtaagcggatgcc

SEQ ID NO: 31 - DNA, 2412 bp, Artificial Sequence
  Enz.2
atgcaccatcatcatcatcatggcggtagcggcatgattgaagtactgcgccaacagctgctggatagcccgcgttcatggcgtgcattcctgcgtcatttagtcgcatctcagcgtgactcatggctacataccgatttacagcacgcgtgcaagacgtttcgtgaacagcctccggaaggctatcctgaagatattggttggctggcagattttattgcgcattgccaggaagcgatcttccgggatccgtggatggtttttgcgtggcgtctacgtccaggtgtttgggagtatgtgcgcatacatgtagaacagctggcggtggaggagctgagcactgatgaatatctgcaagccaaagaacaacttgttggcttaggtgcagaaggtgaagctgttctgacggtggatttcgaagattttcgtccggtgagccagcgtttaaaagacgagagcaccattggtgatggtcttacccatctgaatcgtcatttagcaggtcgcatctggactgatttagcagcaggtcgtagtgctattctggaatttctgggcctgcatcgtctggataaccagaatctgatgctgagcaacggcaataccgattttgactctttacgtcaaaccgtacaatatctgggcaccttaccaagagaaactccgtgggcagagtttcgtgaagacatgcgtcgtcgtggttttgaacccggttggggcaacaccgcgggccgtgttcgcgaaaccatgcgtctgctgatggatctgcttgactctccgagcccagctgccctggagagcttcctggatcgcatcccgatgattagcaacgttctgatcgtgagcattcacggatggtttgcgcaggacaaggttctgggtcgtccggacactggtggtcaggtcgtgtatattctggatcaggcccgtgcactggaacgcgaaatgcgtaaccgcctgcgccaacagggtgttgatgtggagccgcgcattttgattgcgacccgtttaatcccggaaagtgatggcacgacttgtgaccagcgtctggagcctgtccatggtgccgagaatgtgcagattctgcgcgttccgtttcgctatgaggatggtcgtattcacccgcattggatctcacgcttcaaggtttggccgtatcttgaacgctatgcaagggatctggaacgcgaagttaaggccgaattaggtagtcgtccagatctgatcatcggcaactatagcgacggtgggctggttgcaaccatcctgtcagaaaaattaggtgttacgcagtgcaacattgcacatgccctggagaaaagcaagtacccggggtccgatctgcattggccgctgtatgaacaggaccatcactttgcgtgtcagtttaccgcggatctgatcgcgatgaatgcagcagacatcatcgtgacgagcacataccaggaaattgcaggtaatgaccgcgaggttggtcaatatgaatctcaccaggactatactttaccgggcttgtatcgtgtcgagaatggtattgacgtgttcgatagcaagtttaacattgtgagtccgggcgcagatccgagtacgtattttagctatgcccgtcatgaagaacgcttctcgtcgctgtggccagaaatcgaaagtctgctgtttggccgcgaaccaggtccggatattcgtggtgttctcgaagatcctcagaaaccgattattctgtcggtggcccgtatggatcgcatcaagaacctgagcggtctggccgaactgtatggtcggagtgcgcgcttacgtagcctggccaatttggtgatcatcggtggtcatgttgatgtacaggccagtatggatgcagaagaacgcgaagaaatccgtcgtatgcacgagatcatggaccgctaccagctggatggtcagatgcgttgggtgggatcgcatctggataaacgcgtcgtgggcgaattgtatcgtgtagtggcggatggacgtggcgtttttgtgcaaccagccctgtttgaggcgttcggcctgaccgtgattgaggcaatgagcagtggcctgccagtgtttgcgacccgccacggtggtccgctggaaatcatcgaagacggcgttagcggcttccatattgatcccaacgaccctgaagcggtagcagaaaaactggccgacttcctggaagcagcgcgtgaacgtccgaagtattgggaggaaattagccaggcggctcttgcgcgcgtcagcgaacgttacacgtgggagcgctatgcggaacgcttgatgaccatcgcgcgttgcttcggcttttggcgcttcgttctgtcacgcgaatcacaggtcatggaacgctatctgcaaatgttccgccacctgcaatggcgcccgctggctcatgccgtaccgatggag

SEQ ID NO: 32 - protein, 804 aa, Artificial Sequence
  Enz.2
MHHHHHHGGSGMIEVLRQQLLDSPRSWRAFLRHLVASQRDSWLHTDLQHACKTFREQPPEGYPEDIGWLADFIAHCQEAIFRDPWMVFAWRLRPGVWEYVRIHVEQLAVEELSTDEYLQAKEQLVGLGAEGEAVLTVDFEDFRPVSQRLKDESTIGDGLTHLNRHLAGRIWTDLAAGRSAILEFLGLHRLDNQNLMLSNGNTDFDSLRQTVQYLGTLPRETPWAEFREDMRRRGFEPGWGNTAGRVRETMRLLMDLLDSPSPAALESFLDRIPMISNVLIVSIHGWFAQDKVLGRPDTGGQVVYILDQARALEREMRNRLRQQGVDVEPRILIATRLIPESDGTTCDQRLEPVHGAENVQILRVPFRYEDGRIHPHWISRFKVWPYLERYARDLEREVKAELGSRPDLIIGNYSDGGLVATILSEKLGVTQCNIAHALEKSKYPGSDLHWPLYEQDHHFACQFTADLIAMNAADIIVTSTYQEIAGNDREVGQYESHQDYTLPGLYRVENGIDVFDSKFNIVSPGADPSTYFSYARHEERFSSLWPEIESLLFGREPGPDIRGVLEDPQKPIILSVARMDRIKNLSGLAELYGRSARLRSLANLVIIGGHVDVQASMDAEEREEIRRMHEIMDRYQLDGQMRWVGSHLDKRVVGELYRVVADGRGVFVQPALFEAFGLTVIEAMSSGLPVFATRHGGPLEIIEDGVSGFHIDPNDPEAVAEKLADFLEAARERPKYWEEISQAALARVSERYTWERYAERLMTIARCFGFWRFVLSRESQVMERYLQMFRHLQWRPLAHAVPME

SEQ ID NO: 33 - DNA, 1371 bp, Artificial Sequence
  Enz.3
atgccgaacaccaacccgaccaccgttcgtcgtcgtcgtgttatcatgttcccggttccgttcccgggtcacctgaacccgatgctgcagctggctaacgttctgtaccgtcgtggtttcgaaatcaccatcctgcacaccaacttcaacgctccgaaaacctctctgtacccgcacttccagttccgtttcatcctggacaacgacccgcagccggaatggctgcgtaacctgccgaccaccggtccgggtgttggtgctcgtatcccggttatcaacaaacacggtgctgacgaattccgtaaagaactggaaatctgcatgcgtgacaccccgtctgacgaagaagttgcttgcgttatcaccgacgctctgtggtacttcgctcagccggttgctgactctctgaacctgaaacgtctggttctgcagaccggttctctgttcaacttccactgcctggtttgcctgccgaaattcctggaactgggttacctggacccggaaaccaaacaccgtccggacgaaccggttgttggtttcccgatgctgaaagttaaagacatccgtcgtgcttactctcacatccaggaatctaaaccgatcctgatgaaaatggttgaagaaacccgtgcttcttctggtgttatctggaactctgctaaagaactggaagaatctgaactggaaaccatccagcgtgaaatcccggctccgtctttcctgctgccgctgccgaaacactaccgtgcttcttctacctctctgctggacaccgacccgtctaccgctcagtggctggaccagcagccgccgtcttctgttctgtacgttggtttcggttctcagtcttctctggacccggctgacttcctggaaatcgctcgtggtctggttgcttctaaacagtctttcctgtgggctgttcgtccgggtttcgttaaaggttacgaatggatcgaactgctgccggacggtttcctgggtgaaaaaggtcgtatcgttaaatctgctccgcagcaggaagttctggctcacaaagctatcggtgctttctggacccacggtggttggaacggtaccatggaagctgtttgcgaaggtgttccgatgatcttctctgacttcggtctggaccagccgctgaacgctcgttacatgtctgaagttctgcacgttggtgtttacctggaaaacggtttcatccgtggtgaaatcatcaacgctgttcgtcgtgttatggttgacccggaaggtgaagttatgcgtcagaacgctcgtaaactgaaagacaaactggaccgttctatcgctccgggtggttcttcttacgaatctctggaacgtctgcagtcttacatctcttctctg

SEQ ID NO: 34 - DNA, 1371 bp, Artificial Sequence
  Enz.4
atgccgaacaccaacccgaccaccgttcgtcgtcgtcgtgttatcatgttcccggttccgttcccgggtcacctgaacccgatgctgcagctggctaacgttctgtaccgtcgtggtttcgaaatcaccatcctgcacaccaacttcaacgctccgaaaacctctctgtacccgcacttccagttccgtttcatcctggacaacgacccgcagccggaatggctgcgtaacctgccgaccaccggtccgggtgttggtgctcgtatcccggttatcaacaaacacggtgctgacgaattccgtaaagaactggaaatctgcatgcgtgacaccccgtctgacgaagaagttgcttgcgttatcaccgacgctctgtggtacttcgctcagccggttgctgactctctgaacctgaaacgtctggttctgcagaccggttctctgttcaacttccactgcctggtttgcctgccgaaattcctggaactgggttacctggacccggaaaccaaacaccgtccggacgaaccggttgttggtttcccgatgctgaaagttaaagacatccgtcgtgcttactctcacatccaggaatctaaaccgatcctgatgaaaatggttgaagaaacccgtgcttcttctggtgttatctggaactctgctaaagaactggaagaatctgaactggaaaccatccagcgtgaaatcccggctccgtctttcctgctgccgctgccgaaacactaccgtgcttcttctacctctctgctggacaccgacccgtctaccgctcagtggctggaccagcagccgccgtcttctgttctgtacgttggtttcggttctcagtcttctctggacccggctgacttcctggaaatcgctcgtggtctggttgcttctaaacagtctttcctgtgggacgttcgtccgggtttcgttaaaggttacgaatggatcgaactgctgccggacggtttcctgggtgaaaaaggtcgtatcgttaaatctgctccgcagcaggaagttctggctcacaaagctatcggtgctttctggacccacggtggttggaacggtaccatggaagctgtttgcgaaggtgttccgatgatcttctctgacttcggtctggaccagccgctgaacgctcgttacatgtctgaagttctgcacgttggtgtttacctggaaaacggtttcatccgtggtgaaatcatcaacgctgttcgtcgtgttatggttgacccggaaggtgaagttatgcgtcagaacgctcgtaaactgaaagacaaactggaccgttctatcgctccgggtggttcttcttacgaatctctggaacgtctgcagtcttacatctcttctctg

SEQ ID NO: 35 - DNA, 1371 bp, Artificial Sequence
  Enz.5
atgccgaacaccaacccgaccaccgttcgtcgtcgtcgtgttatcatgttcccggttccgttcccgggtcacctgaacccgatgctgcagctggctaacgttctgtaccgtcgtggtttcgaaatcaccatcctgcacaccaacttcaacgctccgaaaacctctctgtacccgcacttccagttccgtttcatcctggacaacgacccgcagccggaatggctgcgtaacctgccgaccaccggtccgggtgttggtgctcgtatcccggttatcaacaaacacggtgctgacgaattccgtaaagaactggaaatctgcatgcgtgacaccccgtctgacgaagaagttgcttgcgttatcaccgacgctctgtggtacttcgctcagccggttgctgactctctgaacctgaaacgtctggttctgcagaccggttctctgttcaacttccactgcctggtttgcctgccgaaattcctggaactgggttacctggacccggaaaccaaacaccgtccggacgaaccggttgttggtttcccgatgctgaaagttaaagacatccgtcgtgcttactctcacatccaggaatctaaaccgatcctgatgaaaatggttgaagaaacccgtgcttcttctggtgttatctggaactctgctaaagaactggaagaatctgaactggaaaccatccagcgtgaaatcccggctccgtctttcctgctgccgctgccgaaacactaccgtgcttcttctacctctctgctggacaccgacccgtctaccgctcagtggctggaccagcagccgccgtcttctgttctgtacgttggtttcggttctcagtcttctctggacccggctgacttcctggaaatcgctcgtggtctggttgcttctaaacagtctttcctgtgggaagttcgtccgggtttcgttaaaggttacgaatggatcgaactgctgccggacggtttcctgggtgaaaaaggtcgtatcgttaaatctgctccgcagcaggaagttctggctcacaaagctatcggtgctttctggacccacggtggttggaacggtaccatggaagctgtttgcgaaggtgttccgatgatcttctctgacttcggtctggaccagccgctgaacgctcgttacatgtctgaagttctgcacgttggtgtttacctggaaaacggtttcatccgtggtgaaatcatcaacgctgttcgtcgtgttatggttgacccggaaggtgaagttatgcgtcagaacgctcgtaaactgaaagacaaactggaccgttctatcgctccgggtggttcttcttacgaatctctggaacgtctgcagtcttacatctcttctctg

SEQ ID NO: 36 - DNA, 1371 bp, Artificial Sequence
  Enz.6
atgccgaacaccaacccgaccaccgttcgtcgtcgtcgtgttatcatgttcccggttccgttcccgggtcacctgaacccgatgctgcagctggctaacgttctgtaccgtcgtggtttcgaaatcaccatcctgcacaccaacttcaacgctccgaaaacctctctgtacccgcacttccagttccgtttcatcctggacaacgacccgcagccggaatggctgcgtaacctgccgaccaccggtccgggtgttggtgctcgtatcccggttatcaacaaacacggtgctgacgaattccgtaaagaactggaaatctgcatgcgtgacaccccgtctgacgaagaagttgcttgcgttatcaccgacgctctgtggtacttcgctcagccggttgctgactctctgaacctgaaacgtctggttctgcagaccggttctctgttcaacttccactgcctggtttgcctgccgaaattcctggaactgggttacctggacccggaaaccaaacaccgtccggacgaaccggttgttggtttcccgatgctgaaagttaaagacatccgtcgtgcttactctcacatccaggaatctaaaccgatcctgatgaaaatggttgaagaaacccgtgcttcttctggtgttatctggaactctgctaaagaactggaagaatctgaactggaaaccatccagcgtgaaatcccggctccgtctttcctgctgccgctgccgaaacactaccgtgcttcttctacctctctgctggacaccgacccgtctaccgctcagtggctggaccagcagccgccgtcttctgttctgtacgttggtttcggttctcagtcttctctggacccggctgacttcctggaaatcgctcgtggtctggttgcttctaaacagtctttcctgtggggtgttcgtccgggtttcgttaaaggttacgaatggatcgaactgctgccggacggtttcctgggtgaaaaaggtcgtatcgttaaatctgctccgcagcaggaagttctggctcacaaagctatcggtgctttctggacccacggtggttggaacggtaccatggaagctgtttgcgaaggtgttccgatgatcttctctgacttcggtctggaccagccgctgaacgctcgttacatgtctgaagttctgcacgttggtgtttacctggaaaacggtttcatccgtggtgaaatcatcaacgctgttcgtcgtgttatggttgacccggaaggtgaagttatgcgtcagaacgctcgtaaactgaaagacaaactggaccgttctatcgctccgggtggttcttcttacgaatctctggaacgtctgcagtcttacatctcttctctg

SEQ ID NO: 37 - DNA, 1371 bp, Artificial Sequence
  Enz.7
atgccgaacaccaacccgaccaccgttcgtcgtcgtcgtgttatcatgttcccggttccgttcccgggtcacctgaacccgatgctgcagctggctaacgttctgtaccgtcgtggtttcgaaatcaccatcctgcacaccaacttcaacgctccgaaaacctctctgtacccgcacttccagttccgtttcatcctggacaacgacccgcagccggaatggctgcgtaacctgccgaccaccggtccgggtgttggtgctcgtatcccggttatcaacaaacacggtgctgacgaattccgtaaagaactggaaatctgcatgcgtgacaccccgtctgacgaagaagttgcttgcgttatcaccgacgctctgtggtacttcgctcagccggttgctgactctctgaacctgaaacgtctggttctgcagaccggttctctgttcaacttccactgcctggtttgcctgccgaaattcctggaactgggttacctggacccggaaaccaaacaccgtccggacgaaccggttgttggtttcccgatgctgaaagttaaagacatccgtcgtgcttactctcacatccaggaatctaaaccgatcctgatgaaaatggttgaagaaacccgtgcttcttctggtgttatctggaactctgctaaagaactggaagaatctgaactggaaaccatccagcgtgaaatcccggctccgtctttcctgctgccgctgccgaaacactaccgtgcttcttctacctctctgctggacaccgacccgtctaccgctcagtggctggaccagcagccgccgtcttctgttctgtacgttggtttcggttctcagtcttctctggacccggctgacttcctggaaatcgctcgtggtctggttgcttctaaacagtctttcctgtggcacgttcgtccgggtttcgttaaaggttacgaatggatcgaactgctgccggacggtttcctgggtgaaaaaggtcgtatcgttaaatctgctccgcagcaggaagttctggctcacaaagctatcggtgctttctggacccacggtggttggaacggtaccatggaagctgtttgcgaaggtgttccgatgatcttctctgacttcggtctggaccagccgctgaacgctcgttacatgtctgaagttctgcacgttggtgtttacctggaaaacggtttcatccgtggtgaaatcatcaacgctgttcgtcgtgttatggttgacccggaaggtgaagttatgcgtcagaacgctcgtaaactgaaagacaaactggaccgttctatcgctccgggtggttcttcttacgaatctctggaacgtctgcagtcttacatctcttctctg

SEQ ID NO: 38 - DNA, 1371 bp, Artificial Sequence
  Enz.8
atgccgaacaccaacccgaccaccgttcgtcgtcgtcgtgttatcatgttcccggttccgttcccgggtcacctgaacccgatgctgcagctggctaacgttctgtaccgtcgtggtttcgaaatcaccatcctgcacaccaacttcaacgctccgaaaacctctctgtacccgcacttccagttccgtttcatcctggacaacgacccgcagccggaatggctgcgtaacctgccgaccaccggtccgggtgttggtgctcgtatcccggttatcaacaaacacggtgctgacgaattccgtaaagaactggaaatctgcatgcgtgacaccccgtctgacgaagaagttgcttgcgttatcaccgacgctctgtggtacttcgctcagccggttgctgactctctgaacctgaaacgtctggttctgcagaccggttctctgttcaacttccactgcctggtttgcctgccgaaattcctggaactgggttacctggacccggaaaccaaacaccgtccggacgaaccggttgttggtttcccgatgctgaaagttaaagacatccgtcgtgcttactctcacatccaggaatctaaaccgatcctgatgaaaatggttgaagaaacccgtgcttcttctggtgttatctggaactctgctaaagaactggaagaatctgaactggaaaccatccagcgtgaaatcccggctccgtctttcctgctgccgctgccgaaacactaccgtgcttcttctacctctctgctggacaccgacccgtctaccgctcagtggctggaccagcagccgccgtcttctgttctgtacgttggtttcggttctcagtcttctctggacccggctgacttcctggaaatcgctcgtggtctggttgcttctaaacagtctttcctgtggatcgttcgtccgggtttcgttaaaggttacgaatggatcgaactgctgccggacggtttcctgggtgaaaaaggtcgtatcgttaaatctgctccgcagcaggaagttctggctcacaaagctatcggtgctttctggacccacggtggttggaacggtaccatggaagctgtttgcgaaggtgttccgatgatcttctctgacttcggtctggaccagccgctgaacgctcgttacatgtctgaagttctgcacgttggtgtttacctggaaaacggtttcatccgtggtgaaatcatcaacgctgttcgtcgtgttatggttgacccggaaggtgaagttatgcgtcagaacgctcgtaaactgaaagacaaactggaccgttctatcgctccgggtggttcttcttacgaatctctggaacgtctgcagtcttacatctcttctctg

SEQ ID NO: 39 - DNA, 1371 bp, Artificial Sequence
  Enz.9
atgccgaacaccaacccgaccaccgttcgtcgtcgtcgtgttatcatgttcccggttccgttcccgggtcacctgaacccgatgctgcagctggctaacgttctgtaccgtcgtggtttcgaaatcaccatcctgcacaccaacttcaacgctccgaaaacctctctgtacccgcacttccagttccgtttcatcctggacaacgacccgcagccggaatggctgcgtaacctgccgaccaccggtccgggtgttggtgctcgtatcccggttatcaacaaacacggtgctgacgaattccgtaaagaactggaaatctgcatgcgtgacaccccgtctgacgaagaagttgcttgcgttatcaccgacgctctgtggtacttcgctcagccggttgctgactctctgaacctgaaacgtctggttctgcagaccggttctctgttcaacttccactgcctggtttgcctgccgaaattcctggaactgggttacctggacccggaaaccaaacaccgtccggacgaaccggttgttggtttcccgatgctgaaagttaaagacatccgtcgtgcttactctcacatccaggaatctaaaccgatcctgatgaaaatggttgaagaaacccgtgcttcttctggtgttatctggaactctgctaaagaactggaagaatctgaactggaaaccatccagcgtgaaatcccggctccgtctttcctgctgccgctgccgaaacactaccgtgcttcttctacctctctgctggacaccgacccgtctaccgctcagtggctggaccagcagccgccgtcttctgttctgtacgttggtttcggttctcagtcttctctggacccggctgacttcctggaaatcgctcgtggtctggttgcttctaaacagtctttcctgtggaaagttcgtccgggtttcgttaaaggttacgaatggatcgaactgctgccggacggtttcctgggtgaaaaaggtcgtatcgttaaatctgctccgcagcaggaagttctggctcacaaagctatcggtgctttctggacccacggtggttggaacggtaccatggaagctgtttgcgaaggtgttccgatgatcttctctgacttcggtctggaccagccgctgaacgctcgttacatgtctgaagttctgcacgttggtgtttacctggaaaacggtttcatccgtggtgaaatcatcaacgctgttcgtcgtgttatggttgacccggaaggtgaagttatgcgtcagaacgctcgtaaactgaaagacaaactggaccgttctatcgctccgggtggttcttcttacgaatctctggaacgtctgcagtcttacatctcttctctg

SEQ ID NO: 40 - DNA, 1371 bp, Artificial Sequence
  Enz.10
atgccgaacaccaacccgaccaccgttcgtcgtcgtcgtgttatcatgttcccggttccgttcccgggtcacctgaacccgatgctgcagctggctaacgttctgtaccgtcgtggtttcgaaatcaccatcctgcacaccaacttcaacgctccgaaaacctctctgtacccgcacttccagttccgtttcatcctggacaacgacccgcagccggaatggctgcgtaacctgccgaccaccggtccgggtgttggtgctcgtatcccggttatcaacaaacacggtgctgacgaattccgtaaagaactggaaatctgcatgcgtgacaccccgtctgacgaagaagttgcttgcgttatcaccgacgctctgtggtacttcgctcagccggttgctgactctctgaacctgaaacgtctggttctgcagaccggttctctgttcaacttccactgcctggtttgcctgccgaaattcctggaactgggttacctggacccggaaaccaaacaccgtccggacgaaccggttgttggtttcccgatgctgaaagttaaagacatccgtcgtgcttactctcacatccaggaatctaaaccgatcctgatgaaaatggttgaagaaacccgtgcttcttctggtgttatctggaactctgctaaagaactggaagaatctgaactggaaaccatccagcgtgaaatcccggctccgtctttcctgctgccgctgccgaaacactaccgtgcttcttctacctctctgctggacaccgacccgtctaccgctcagtggctggaccagcagccgccgtcttctgttctgtacgttggtttcggttctcagtcttctctggacccggctgacttcctggaaatcgctcgtggtctggttgcttctaaacagtctttcctgtggatggttcgtccgggtttcgttaaaggttacgaatggatcgaactgctgccggacggtttcctgggtgaaaaaggtcgtatcgttaaatctgctccgcagcaggaagttctggctcacaaagctatcggtgctttctggacccacggtggttggaacggtaccatggaagctgtttgcgaaggtgttccgatgatcttctctgacttcggtctggaccagccgctgaacgctcgttacatgtctgaagttctgcacgttggtgtttacctggaaaacggtttcatccgtggtgaaatcatcaacgctgttcgtcgtgttatggttgacccggaaggtgaagttatgcgtcagaacgctcgtaaactgaaagacaaactggaccgttctatcgctccgggtggttcttcttacgaatctctggaacgtctgcagtcttacatctcttctctg

SEQ ID NO: 41 - DNA, 1371 bp, Artificial Sequence
  Enz.11
atgccgaacaccaacccgaccaccgttcgtcgtcgtcgtgttatcatgttcccggttccgttcccgggtcacctgaacccgatgctgcagctggctaacgttctgtaccgtcgtggtttcgaaatcaccatcctgcacaccaacttcaacgctccgaaaacctctctgtacccgcacttccagttccgtttcatcctggacaacgacccgcagccggaatggctgcgtaacctgccgaccaccggtccgggtgttggtgctcgtatcccggttatcaacaaacacggtgctgacgaattccgtaaagaactggaaatctgcatgcgtgacaccccgtctgacgaagaagttgcttgcgttatcaccgacgctctgtggtacttcgctcagccggttgctgactctctgaacctgaaacgtctggttctgcagaccggttctctgttcaacttccactgcctggtttgcctgccgaaattcctggaactgggttacctggacccggaaaccaaacaccgtccggacgaaccggttgttggtttcccgatgctgaaagttaaagacatccgtcgtgcttactctcacatccaggaatctaaaccgatcctgatgaaaatggttgaagaaacccgtgcttcttctggtgttatctggaactctgctaaagaactggaagaatctgaactggaaaccatccagcgtgaaatcccggctccgtctttcctgctgccgctgccgaaacactaccgtgcttcttctacctctctgctggacaccgacccgtctaccgctcagtggctggaccagcagccgccgtcttctgttctgtacgttggtttcggttctcagtcttctctggacccggctgacttcctggaaatcgctcgtggtctggttgcttctaaacagtctttcctgtggaacgttcgtccgggtttcgttaaaggttacgaatggatcgaactgctgccggacggtttcctgggtgaaaaaggtcgtatcgttaaatctgctccgcagcaggaagttctggctcacaaagctatcggtgctttctggacccacggtggttggaacggtaccatggaagctgtttgcgaaggtgttccgatgatcttctctgacttcggtctggaccagccgctgaacgctcgttacatgtctgaagttctgcacgttggtgtttacctggaaaacggtttcatccgtggtgaaatcatcaacgctgttcgtcgtgttatggttgacccggaaggtgaagttatgcgtcagaacgctcgtaaactgaaagacaaactggaccgttctatcgctccgggtggttcttcttacgaatctctggaacgtctgcagtcttacatctcttctctg

SEQ ID NO: 42 - DNA, 1371 bp, Artificial Sequence
  Enz.12
atgccgaacaccaacccgaccaccgttcgtcgtcgtcgtgttatcatgttcccggttccgttcccgggtcacctgaacccgatgctgcagctggctaacgttctgtaccgtcgtggtttcgaaatcaccatcctgcacaccaacttcaacgctccgaaaacctctctgtacccgcacttccagttccgtttcatcctggacaacgacccgcagccggaatggctgcgtaacctgccgaccaccggtccgggtgttggtgctcgtatcccggttatcaacaaacacggtgctgacgaattccgtaaagaactggaaatctgcatgcgtgacaccccgtctgacgaagaagttgcttgcgttatcaccgacgctctgtggtacttcgctcagccggttgctgactctctgaacctgaaacgtctggttctgcagaccggttctctgttcaacttccactgcctggtttgcctgccgaaattcctggaactgggttacctggacccggaaaccaaacaccgtccggacgaaccggttgttggtttcccgatgctgaaagttaaagacatccgtcgtgcttactctcacatccaggaatctaaaccgatcctgatgaaaatggttgaagaaacccgtgcttcttctggtgttatctggaactctgctaaagaactggaagaatctgaactggaaaccatccagcgtgaaatcccggctccgtctttcctgctgccgctgccgaaacactaccgtgcttcttctacctctctgctggacaccgacccgtctaccgctcagtggctggaccagcagccgccgtcttctgttctgtacgttggtttcggttctcagtcttctctggacccggctgacttcctggaaatcgctcgtggtctggttgcttctaaacagtctttcctgtggccggttcgtccgggtttcgttaaaggttacgaatggatcgaactgctgccggacggtttcctgggtgaaaaaggtcgtatcgttaaatctgctccgcagcaggaagttctggctcacaaagctatcggtgctttctggacccacggtggttggaacggtaccatggaagctgtttgcgaaggtgttccgatgatcttctctgacttcggtctggaccagccgctgaacgctcgttacatgtctgaagttctgcacgttggtgtttacctggaaaacggtttcatccgtggtgaaatcatcaacgctgttcgtcgtgttatggttgacccggaaggtgaagttatgcgtcagaacgctcgtaaactgaaagacaaactggaccgttctatcgctccgggtggttcttcttacgaatctctggaacgtctgcagtcttacatctcttctctg

SEQ ID NO: 43 - DNA, 1371 bp, Artificial Sequence
  Enz.13
atgccgaacaccaacccgaccaccgttcgtcgtcgtcgtgttatcatgttcccggttccgttcccgggtcacctgaacccgatgctgcagctggctaacgttctgtaccgtcgtggtttcgaaatcaccatcctgcacaccaacttcaacgctccgaaaacctctctgtacccgcacttccagttccgtttcatcctggacaacgacccgcagccggaatggctgcgtaacctgccgaccaccggtccgggtgttggtgctcgtatcccggttatcaacaaacacggtgctgacgaattccgtaaagaactggaaatctgcatgcgtgacaccccgtctgacgaagaagttgcttgcgttatcaccgacgctctgtggtacttcgctcagccggttgctgactctctgaacctgaaacgtctggttctgcagaccggttctctgttcaacttccactgcctggtttgcctgccgaaattcctggaactgggttacctggacccggaaaccaaacaccgtccggacgaaccggttgttggtttcccgatgctgaaagttaaagacatccgtcgtgcttactctcacatccaggaatctaaaccgatcctgatgaaaatggttgaagaaacccgtgcttcttctggtgttatctggaactctgctaaagaactggaagaatctgaactggaaaccatccagcgtgaaatcccggctccgtctttcctgctgccgctgccgaaacactaccgtgcttcttctacctctctgctggacaccgacccgtctaccgctcagtggctggaccagcagccgccgtcttctgttctgtacgttggtttcggttctcagtcttctctggacccggctgacttcctggaaatcgctcgtggtctggttgcttctaaacagtctttcctgtggtctgttcgtccgggtttcgttaaaggttacgaatggatcgaactgctgccggacggtttcctgggtgaaaaaggtcgtatcgttaaatctgctccgcagcaggaagttctggctcacaaagctatcggtgctttctggacccacggtggttggaacggtaccatggaagctgtttgcgaaggtgttccgatgatcttctctgacttcggtctggaccagccgctgaacgctcgttacatgtctgaagttctgcacgttggtgtttacctggaaaacggtttcatccgtggtgaaatcatcaacgctgttcgtcgtgttatggttgacccggaaggtgaagttatgcgtcagaacgctcgtaaactgaaagacaaactggaccgttctatcgctccgggtggttcttcttacgaatctctggaacgtctgcagtcttacatctcttctctg

SEQ ID NO: 44 - DNA, 1371 bp, Artificial Sequence
  Enz.14
atgccgaacaccaacccgaccaccgttcgtcgtcgtcgtgttatcatgttcccggttccgttcccgggtcacctgaacccgatgctgcagctggctaacgttctgtaccgtcgtggtttcgaaatcaccatcctgcacaccaacttcaacgctccgaaaacctctctgtacccgcacttccagttccgtttcatcctggacaacgacccgcagccggaatggctgcgtaacctgccgaccaccggtccgggtgttggtgctcgtatcccggttatcaacaaacacggtgctgacgaattccgtaaagaactggaaatctgcatgcgtgacaccccgtctgacgaagaagttgcttgcgttatcaccgacgctctgtggtacttcgctcagccggttgctgactctctgaacctgaaacgtctggttctgcagaccggttctctgttcaacttccactgcctggtttgcctgccgaaattcctggaactgggttacctggacccggaaaccaaacaccgtccggacgaaccggttgttggtttcccgatgctgaaagttaaagacatccgtcgtgcttactctcacatccaggaatctaaaccgatcctgatgaaaatggttgaagaaacccgtgcttcttctggtgttatctggaactctgctaaagaactggaagaatctgaactggaaaccatccagcgtgaaatcccggctccgtctttcctgctgccgctgccgaaacactaccgtgcttcttctacctctctgctggacaccgacccgtctaccgctcagtggctggaccagcagccgccgtcttctgttctgtacgttggtttcggttctcagtcttctctggacccggctgacttcctggaaatcgctcgtggtctggttgcttctaaacagtctttcctgtgggttgttcgtccgggtttcgttaaaggttacgaatggatcgaactgctgccggacggtttcctgggtgaaaaaggtcgtatcgttaaatctgctccgcagcaggaagttctggctcacaaagctatcggtgctttctggacccacggtggttggaacggtaccatggaagctgtttgcgaaggtgttccgatgatcttctctgacttcggtctggaccagccgctgaacgctcgttacatgtctgaagttctgcacgttggtgtttacctggaaaacggtttcatccgtggtgaaatcatcaacgctgttcgtcgtgttatggttgacccggaaggtgaagttatgcgtcagaacgctcgtaaactgaaagacaaactggaccgttctatcgctccgggtggttcttcttacgaatctctggaacgtctgcagtcttacatctcttctctg

SEQ ID NO: 45 - DNA, 1371 bp, Artificial Sequence
  Enz.15
atgccgaacaccaacccgaccaccgttcgtcgtcgtcgtgttatcatgttcccggttccgttcccgggtcacctgaacccgatgctgcagctggctaacgttctgtaccgtcgtggtttcgaaatcaccatcctgcacaccaacttcaacgctccgaaaacctctctgtacccgcacttccagttccgtttcatcctggacaacgacccgcagccggaatggctgcgtaacctgccgaccaccggtccgggtgttggtgctcgtatcccggttatcaacaaacacggtgctgacgaattccgtaaagaactggaaatctgcatgcgtgacaccccgtctgacgaagaagttgcttgcgttatcaccgacgctctgtggtacttcgctcagccggttgctgactctctgaacctgaaacgtctggttctgcagaccggttctctgttcaacttccactgcctggtttgcctgccgaaattcctggaactgggttacctggacccggaaaccaaacaccgtccggacgaaccggttgttggtttcccgatgctgaaagttaaagacatccgtcgtgcttactctcacatccaggaatctaaaccgatcctgatgaaaatggttgaagaaacccgtgcttcttctggtgttatctggaactctgctaaagaactggaagaatctgaactggaaaccatccagcgtgaaatcccggctccgtctttcctgctgccgctgccgaaacactaccgtgcttcttctacctctctgctggacaccgacccgtctaccgctcagtggctggaccagcagccgccgtcttctgttctgtacgttggtttcggttctcagtcttctctggacccggctgacttcctggaaatcgctcgtggtctggttgcttctaaacagtctttcctgtggtgggttcgtccgggtttcgttaaaggttacgaatggatcgaactgctgccggacggtttcctgggtgaaaaaggtcgtatcgttaaatctgctccgcagcaggaagttctggctcacaaagctatcggtgctttctggacccacggtggttggaacggtaccatggaagctgtttgcgaaggtgttccgatgatcttctctgacttcggtctggaccagccgctgaacgctcgttacatgtctgaagttctgcacgttggtgtttacctggaaaacggtttcatccgtggtgaaatcatcaacgctgttcgtcgtgttatggttgacccggaaggtgaagttatgcgtcagaacgctcgtaaactgaaagacaaactggaccgttctatcgctccgggtggttcttcttacgaatctctggaacgtctgcagtcttacatctcttctctg

SEQ ID NO: 46 - DNA, 29 bp, Artificial Sequence
  GT029-R12Q-F
gcgtcgtcagcgtgttattatgtttccgg

SEQ ID NO: 47 - DNA, 33 bp, Artificial Sequence
  GT029-R12Q-R
cataataacacgctgacgacgcacggtagttgg

SEQ ID NO: 48 - DNA, 30 bp, Artificial Sequence
  GT029-V14I-F
cgtcgtatcattatgtttccggttccgttc

SEQ ID NO: 49 - DNA, 33 bp, Artificial Sequence
  GT029-V14I-R
gaaacataatgatacgacgacgacgcacggtag

SEQ ID NO: 50 - DNA, 31 bp, Artificial Sequence
  GT029-E99L-F
cgcggatctattccgtaaggagctggaaatc

SEQ ID NO: 51 - DNA, 32 bp, Artificial Sequence
  GT029-E99L-R
ccttacggaatagatccgcgccgtgtttgtta

SEQ ID NO: 52 - DNA, 29 bp, Artificial Sequence
  GT029-A118S-F
ggaagttagttgcgtgattaccgatgcgc

SEQ ID NO: 53 - DNA, 34 bp, Artificial Sequence
  GT029-A118S-R
gtaatcacgcaactaacttcctcgtcactcggag

SEQ ID NO: 54 - DNA, 31 bp, Artificial Sequence
  GT029-S194P-F
cgcgcgtatccgcacattcaagaatcgaaac

SEQ ID NO: 55 - DNA, 31 bp, Artificial Sequence
  GT029-S194P-R
cttgaatgtgcggatacgcgcgacggatatc

SEQ ID NO: 56 - DNA, 31 bp, Artificial Sequence
  GT029-T254G-F
cttcgagcggtagcctgctggatactgatcc

SEQ ID NO: 57 - DNA, 31 bp, Artificial Sequence
  GT029-T254G-R
cagcaggctaccgctcgaagccctataatgc

SEQ ID NO: 58 - DNA, 33 bp, Artificial Sequence
  GT029-L257A-F
gcactagcctggcggatactgatccgagcaccg

SEQ ID NO: 59 - DNA, 34 bp, Artificial Sequence
  GT029-L257A-R
cggatcagtatccgccaggctagtgctcgaagcc

SEQ ID NO: 60 - DNA, 33 bp, Artificial Sequence
  GT029-E418D-F
gttgaccctgacggtgaggttatgcgccaaaac

SEQ ID NO: 61 - DNA, 27 bp, Artificial Sequence
  GT029-E418D-R
cctcaccgtcagggtcaaccatcacac

SEQ ID NO: 62 - DNA, 30 bp, Artificial Sequence
  GT029-Q451E-F
gaacgcctggagagctatattagcagcctg

SEQ ID NO: 63 - DNA, 33 bp, Artificial Sequence
  GT029-Q451E-R
ctaatatagctctccaggcgttccaggctctcg

SEQ ID NO: 64 - DNA, 30 bp, Artificial Sequence
  GT029-S455R-F
gagctatattcgcagcctgtaagcttgcgg

SEQ ID NO: 65 - DNA, 34 bp, Artificial Sequence
  GT029-S455R-R
cttacaggctgcgaatatagctctgcaggcgttc

SEQ ID NO: 66 - DNA, 28 bp, Artificial Sequence
  GT029-Q265E-F
ccgccgaatggctggaccagcagccgcc

SEQ ID NO: 67 - DNA, 33 bp, Artificial Sequence
  GT029-Q265E-R
gtccagccattcggcggtgctcggatcagtatc

SEQ ID NO: 68 - DNA, 31 bp, Artificial Sequence
  GT029-P271A-F
gaccagcaggcgccgagcagcgtgctgtacg

SEQ ID NO: 69 - DNA, 31 bp, Artificial Sequence
  GT029-P271A-R
ctgctcggcgcctgctggtccagccattggg

SEQ ID NO: 70 - DNA, 30 bp, Artificial Sequence
  GT029-R333K-F
gaaaaaggtaagatcgtgaagtctgctccg

SEQ ID NO: 71 - DNA, 32 bp, Artificial Sequence
  GT029-R333K-R
cttcacgatcttacctttttcacccagaaaac

SEQ ID NO: 72 - DNA, 32 bp, Artificial Sequence
  GT029-K347P-F
ctggcgcaccctgcgattggtgcgttctggac

SEQ ID NO: 73 - DNA, 30 bp, Artificial Sequence
  GT029-K347P-R
accaatcgcagggtgcgccagcacttcttg

SEQ ID NO: 74 - DNA, 32 bp, Artificial Sequence
  GT029-L378G-F
gatttcggtggtgatcagccgctgaacgcgcg

SEQ ID NO: 75 - DNA, 31 bp, Artificial Sequence
  GT029-L378G-R
cggctgatcaccaccgaaatcgctaaagatc

SEQ ID NO: 76 - DNA, 40 bp, Artificial Sequence
  GT029-Q265E-P271A-F
cgaatggctggaccagcaggcgccgagcagcgtgctgtac

SEQ ID NO: 77 - DNA, 42 bp, Artificial Sequence
  GT029-Q265E-P271A-R
gcgcctgctggtccagccattcggcggtgctcggatcagtat

SEQ ID NO: 78 - DNA, 65 bp, Artificial Sequence
  GT029-R333K-K347P-F
aagatcgtgaagtctgctccgcaacaagaagtgctggcgcaccctgcgattggtgcgttctggac

SEQ ID NO: 79 - DNA, 60 bp, Artificial Sequence
  GT029-R333K-K347P-R
agggtgcgccagcacttcttgttgcggagcagacttcacgatcttacctttttcacccag

SEQ ID NO: 80 - DNA, 40 bp, Artificial Sequence; identical to SEQ ID NO: 76
  GT029-Q265E-P271A-F

SEQ ID NO: 81 - DNA, 31 bp, Artificial Sequence; identical to SEQ ID NO: 75
  GT029-L378G-R

SEQ ID NO: 82 - DNA, 32 bp, Artificial Sequence; identical to SEQ ID NO: 74
  GT029-L378G-F

SEQ ID NO: 83 - DNA, 42 bp, Artificial Sequence; identical to SEQ ID NO: 77
  GT029-Q265E-P271A-R

SEQ ID NO: 84 - DNA, 65 bp, Artificial Sequence; identical to SEQ ID NO: 78
  GT029-R333K-K347P-F

SEQ ID NO: 85 - DNA, 42 bp, Artificial Sequence; identical to SEQ ID NO: 77
  GT029-Q265E-P271A-R

SEQ ID NO: 86 - DNA, 40 bp, Artificial Sequence; identical to SEQ ID NO: 76
  GT029-Q265E-P271A-F

SEQ ID NO: 87 - DNA, 60 bp, Artificial Sequence; identical to SEQ ID NO: 79
  GT029-R333K-K347P-R

SEQ ID NO: 88 - DNA, 32 bp, Artificial Sequence; identical to SEQ ID NO: 74
  GT029-L378G-F

SEQ ID NO: 89 - DNA, 31 bp, Artificial Sequence; identical to SEQ ID NO: 75
  GT029-L378G-R

SEQ ID NO: 90 - DNA, 19 bp, Artificial Sequence
  Km-F
gcccgacattatcgcgagc

SEQ ID NO: 91 - DNA, 19 bp, Artificial Sequence
  Km-R
gggtataaatgggctcgcg

SEQ ID NO: 92 - DNA, 1371 bp, Artificial Sequence
  Enz.16
atgccgaacaccaacccgaccaccgttcgtcgtcagcgtgttatcatgttcccggttccgttcccgggtcacctgaacccgatgctgcagctggctaacgttctgtaccgtcgtggtttcgaaatcaccatcctgcacaccaacttcaacgctccgaaaacctctctgtacccgcacttccagttccgtttcatcctggacaacgacccgcagccggaatggctgcgtaacctgccgaccaccggtccgggtgttggtgctcgtatcccggttatcaacaaacacggtgctgacgaattccgtaaagaactggaaatctgcatgcgtgacaccccgtctgacgaagaagttgcttgcgttatcaccgacgctctgtggtacttcgctcagccggttgctgactctctgaacctgaaacgtctggttctgcagaccggttctctgttcaacttccactgcctggtttgcctgccgaaattcctggaactgggttacctggacccggaaaccaaacaccgtccggacgaaccggttgttggtttcccgatgctgaaagttaaagacatccgtcgtgcttactctcacatccaggaatctaaaccgatcctgatgaaaatggttgaagaaacccgtgcttcttctggtgttatctggaactctgctaaagaactggaagaatctgaactggaaaccatccagcgtgaaatcccggctccgtctttcctgctgccgctgccgaaacactaccgtgcttcttctacctctctgctggacaccgacccgtctaccgctcagtggctggaccagcagccgccgtcttctgttctgtacgttggtttcggttctcagtcttctctggacccggctgacttcctggaaatcgctcgtggtctggttgcttctaaacagtctttcctgtggaacgttcgtccgggtttcgttaaaggttacgaatggatcgaactgctgccggacggtttcctgggtgaaaaaggtcgtatcgttaaatctgctccgcagcaggaagttctggctcacaaagctatcggtgctttctggacccacggtggttggaacggtaccatggaagctgtttgcgaaggtgttccgatgatcttctctgacttcggtctggaccagccgctgaacgctcgttacatgtctgaagttctgcacgttggtgtttacctggaaaacggtttcatccgtggtgaaatcatcaacgctgttcgtcgtgttatggttgacccggaaggtgaagttatgcgtcagaacgctcgtaaactgaaagacaaactggaccgttctatcgctccgggtggttcttcttacgaatctctggaacgtctgcagtcttacatctcttctctg

SEQ ID NO: 93 - DNA, 1371 bp, Artificial Sequence
  Enz.17
atgccgaacaccaacccgaccaccgttcgtcgtcgtcgtatcatcatgttcccggttccgttcccgggtcacctgaacccgatgctgcagctggctaacgttctgtaccgtcgtggtttcgaaatcaccatcctgcacaccaacttcaacgctccgaaaacctctctgtacccgcacttccagttccgtttcatcctggacaacgacccgcagccggaatggctgcgtaacctgccgaccaccggtccgggtgttggtgctcgtatcccggttatcaacaaacacggtgctgacgaattccgtaaagaactggaaatctgcatgcgtgacaccccgtctgacgaagaagttgcttgcgttatcaccgacgctctgtggtacttcgctcagccggttgctgactctctgaacctgaaacgtctggttctgcagaccggttctctgttcaacttccactgcctggtttgcctgccgaaattcctggaactgggttacctggacccggaaaccaaacaccgtccggacgaaccggttgttggtttcccgatgctgaaagttaaagacatccgtcgtgcttactctcacatccaggaatctaaaccgatcctgatgaaaatggttgaagaaacccgtgcttcttctggtgttatctggaactctgctaaagaactggaagaatctgaactggaaaccatccagcgtgaaatcccggctccgtctttcctgctgccgctgccgaaacactaccgtgcttcttctacctctctgctggacaccgacccgtctaccgctcagtggctggaccagcagccgccgtcttctgttctgtacgttggtttcggttctcagtcttctctggacccggctgacttcctggaaatcgctcgtggtctggttgcttctaaacagtctttcctgtggaacgttcgtccgggtttcgttaaaggttacgaatggatcgaactgctgccggacggtttcctgggtgaaaaaggtcgtatcgttaaatctgctccgcagcaggaagttctggctcacaaagctatcggtgctttctggacccacggtggttggaacggtaccatggaagctgtttgcgaaggtgttccgatgatcttctctgacttcggtctggaccagccgctgaacgctcgttacatgtctgaagttctgcacgttggtgtttacctggaaaacggtttcatccgtggtgaaatcatcaacgctgttcgtcgtgttatggttgacccggaaggtgaagttatgcgtcagaacgctcgtaaactgaaagacaaactggaccgttctatcgctccgggtggttcttcttacgaatctctggaacgtctgcagtcttacatctcttctctg

SEQ ID NO: 94 - DNA, 1371 bp, Artificial Sequence
  Enz.18
atgccgaacaccaacccgaccaccgttcgtcgtcgtcgtgttatcatgttcccggttccgttcccgggtcacctgaacccgatgctgcagctggctaacgttctgtaccgtcgtggtttcgaaatcaccatcctgcacaccaacttcaacgctccgaaaacctctctgtacccgcacttccagttccgtttcatcctggacaacgacccgcagccggaatggctgcgtaacctgccgaccaccggtccgggtgttggtgctcgtatcccggttatcaacaaacacggtgctgacctgttccgtaaagaactggaaatctgcatgcgtgacaccccgtctgacgaagaagttgcttgcgttatcaccgacgctctgtggtacttcgctcagccggttgctgactctctgaacctgaaacgtctggttctgcagaccggttctctgttcaacttccactgcctggtttgcctgccgaaattcctggaactgggttacctggacccggaaaccaaacaccgtccggacgaaccggttgttggtttcccgatgctgaaagttaaagacatccgtcgtgcttactctcacatccaggaatctaaaccgatcctgatgaaaatggttgaagaaacccgtgcttcttctggtgttatctggaactctgctaaagaactggaagaatctgaactggaaaccatccagcgtgaaatcccggctccgtctttcctgctgccgctgccgaaacactaccgtgcttcttctacctctctgctggacaccgacccgtctaccgctcagtggctggaccagcagccgccgtcttctgttctgtacgttggtttcggttctcagtcttctctggacccggctgacttcctggaaatcgctcgtggtctggttgcttctaaacagtctttcctgtggaacgttcgtccgggtttcgttaaaggttacgaatggatcgaactgctgccggacggtttcctgggtgaaaaaggtcgtatcgttaaatctgctccgcagcaggaagttctggctcacaaagctatcggtgctttctggacccacggtggttggaacggtaccatggaagctgtttgcgaaggtgttccgatgatcttctctgacttcggtctggaccagccgctgaacgctcgttacatgtctgaagttctgcacgttggtgtttacctggaaaacggtttcatccgtggtgaaatcatcaacgctgttcgtcgtgttatggttgacccggaaggtgaagttatgcgtcagaacgctcgtaaactgaaagacaaactggaccgttctatcgctccgggtggttcttcttacgaatctctggaacgtctgcagtcttacatctcttctctg

SEQ ID NO: 95 - DNA, 1371 bp, Artificial Sequence
  Enz.19
atgccgaacaccaacccgaccaccgttcgtcgtcgtcgtgttatcatgttcccggttccgttcccgggtcacctgaacccgatgctgcagctggctaacgttctgtaccgtcgtggtttcgaaatcaccatcctgcacaccaacttcaacgctccgaaaacctctctgtacccgcacttccagttccgtttcatcctggacaacgacccgcagccggaatggctgcgtaacctgccgaccaccggtccgggtgttggtgctcgtatcccggttatcaacaaacacggtgctgacgaattccgtaaagaactggaaatctgcatgcgtgacaccccgtctgacgaagaagtttcttgcgttatcaccgacgctctgtggtacttcgctcagccggttgctgactctctgaacctgaaacgtctggttctgcagaccggttctctgttcaacttccactgcctggtttgcctgccgaaattcctggaactgggttacctggacccggaaaccaaacaccgtccggacgaaccggttgttggtttcccgatgctgaaagttaaagacatccgtcgtgcttactctcacatccaggaatctaaaccgatcctgatgaaaatggttgaagaaacccgtgcttcttctggtgttatctggaactctgctaaagaactggaagaatctgaactggaaaccatccagcgtgaaatcccggctccgtctttcctgctgccgctgccgaaacactaccgtgcttcttctacctctctgctggacaccgacccgtctaccgctcagtggctggaccagcagccgccgtcttctgttctgtacgttggtttcggttctcagtcttctctggacccggctgacttcctggaaatcgctcgtggtctggttgcttctaaacagtctttcctgtggaacgttcgtccgggtttcgttaaaggttacgaatggatcgaactgctgccggacggtttcctgggtgaaaaaggtcgtatcgttaaatctgctccgcagcaggaagttctggctcacaaagctatcggtgctttctggacccacggtggttggaacggtaccatggaagctgtttgcgaaggtgttccgatgatcttctctgacttcggtctggaccagccgctgaacgctcgttacatgtctgaagttctgcacgttggtgtttacctggaaaacggtttcatccgtggtgaaatcatcaacgctgttcgtcgtgttatggttgacccggaaggtgaagttatgcgtcagaacgctcgtaaactgaaagacaaactggaccgttctatcgctccgggtggttcttcttacgaatctctggaacgtctgcagtcttacatctcttctctg

SEQ ID NO: 96 - DNA, 1371 bp, Artificial Sequence
  Enz.20
atgccgaacaccaacccgaccaccgttcgtcgtcgtcgtgttatcatgttcccggttccgttcccgggtcacctgaacccgatgctgcagctggctaacgttctgtaccgtcgtggtttcgaaatcaccatcctgcacaccaacttcaacgctccgaaaacctctctgtacccgcacttccagttccgtttcatcctggacaacgacccgcagccggaatggctgcgtaacctgccgaccaccggtccgggtgttggtgctcgtatcccggttatcaacaaacacggtgctgacgaattccgtaaagaactggaaatctgcatgcgtgacaccccgtctgacgaagaagttgcttgcgttatcaccgacgctctgtggtacttcgctcagccggttgctgactctctgaacctgaaacgtctggttctgcagaccggttctctgttcaacttccactgcctggtttgcctgccgaaattcctggaactgggttacctggacccggaaaccaaacaccgtccggacgaaccggttgttggtttcccgatgctgaaagttaaagacatccgtcgtgcttacccgcacatccaggaatctaaaccgatcctgatgaaaatggttgaagaaacccgtgcttcttctggtgttatctggaactctgctaaagaactggaagaatctgaactggaaaccatccagcgtgaaatcccggctccgtctttcctgctgccgctgccgaaacactaccgtgcttcttctacctctctgctggacaccgacccgtctaccgctcagtggctggaccagcagccgccgtcttctgttctgtacgttggtttcggttctcagtcttctctggacccggctgacttcctggaaatcgctcgtggtctggttgcttctaaacagtctttcctgtggaacgttcgtccgggtttcgttaaaggttacgaatggatcgaactgctgccggacggtttcctgggtgaaaaaggtcgtatcgttaaatctgctccgcagcaggaagttctggctcacaaagctatcggtgctttctggacccacggtggttggaacggtaccatggaagctgtttgcgaaggtgttccgatgatcttctctgacttcggtctggaccagccgctgaacgctcgttacatgtctgaagttctgcacgttggtgtttacctggaaaacggtttcatccgtggtgaaatcatcaacgctgttcgtcgtgttatggttgacccggaaggtgaagttatgcgtcagaacgctcgtaaactgaaagacaaactggaccgttctatcgctccgggtggttcttcttacgaatctctggaacgtctgcagtcttacatctcttctctg

SEQ ID NO: 97 - DNA, 1371 bp, Artificial Sequence
  Enz.21
atgccgaacaccaacccgaccaccgttcgtcgtcgtcgtgttatcatgttcccggttccgttcccgggtcacctgaacccgatgctgcagctggctaacgttctgtaccgtcgtggtttcgaaatcaccatcctgcacaccaacttcaacgctccgaaaacctctctgtacccgcacttccagttccgtttcatcctggacaacgacccgcagccggaatggctgcgtaacctgccgaccaccggtccgggtgttggtgctcgtatcccggttatcaacaaacacggtgctgacgaattccgtaaagaactggaaatctgcatgcgtgacaccccgtctgacgaagaagttgcttgcgttatcaccgacgctctgtggtacttcgctcagccggttgctgactctctgaacctgaaacgtctggttctgcagaccggttctctgttcaacttccactgcctggtttgcctgccgaaattcctggaactgggttacctggacccggaaaccaaacaccgtccggacgaaccggttgttggtttcccgatgctgaaagttaaagacatccgtcgtgcttactctcacatccaggaatctaaaccgatcctgatgaaaatggttgaagaaacccgtgcttcttctggtgttatctggaactctgctaaagaactggaagaatctgaactggaaaccatccagcgtgaaatcccggctccgtctttcctgctgccgctgccgaaacactaccgtgcttcttctggttctctgctggacaccgacccgtctaccgctcagtggctggaccagcagccgccgtcttctgttctgtacgttggtttcggttctcagtcttctctggacccggctgacttcctggaaatcgctcgtggtctggttgcttctaaacagtctttcctgtggaacgttcgtccgggtttcgttaaaggttacgaatggatcgaactgctgccggacggtttcctgggtgaaaaaggtcgtatcgttaaatctgctccgcagcaggaagttctggctcacaaagctatcggtgctttctggacccacggtggttggaacggtaccatggaagctgtttgcgaaggtgttccgatgatcttctctgacttcggtctggaccagccgctgaacgctcgttacatgtctgaagttctgcacgttggtgtttacctggaaaacggtttcatccgtggtgaaatcatcaacgctgttcgtcgtgttatggttgacccggaaggtgaagttatgcgtcagaacgctcgtaaactgaaagacaaactggaccgttctatcgctccgggtggttcttcttacgaatctctggaacgtctgcagtcttacatctcttctctg

SEQ ID NO: 98 - DNA, 1371 bp, Artificial Sequence
  Enz.22
atgccgaacaccaacccgaccaccgttcgtcgtcgtcgtgttatcatgttcccggttccgttcccgggtcacctgaacccgatgctgcagctggctaacgttctgtaccgtcgtggtttcgaaatcaccatcctgcacaccaacttcaacgctccgaaaacctctctgtacccgcacttccagttccgtttcatcctggacaacgacccgcagccggaatggctgcgtaacctgccgaccaccggtccgggtgttggtgctcgtatcccggttatcaacaaacacggtgctgacgaattccgtaaagaactggaaatctgcatgcgtgacaccccgtctgacgaagaagttgcttgcgttatcaccgacgctctgtggtacttcgctcagccggttgctgactctctgaacctgaaacgtctggttctgcagaccggttctctgttcaacttccactgcctggtttgcctgccgaaattcctggaactgggttacctggacccggaaaccaaacaccgtccggacgaaccggttgttggtttcccgatgctgaaagttaaagacatccgtcgtgcttactctcacatccaggaatctaaaccgatcctgatgaaaatggttgaagaaacccgtgcttcttctggtgttatctggaactctgctaaagaactggaagaatctgaactggaaaccatccagcgtgaaatcccggctccgtctttcctgctgccgctgccgaaacactaccgtgcttcttctacctctctggctgacaccgacccgtctaccgctcagtggctggaccagcagccgccgtcttctgttctgtacgttggtttcggttctcagtcttctctggacccggctgacttcctggaaatcgctcgtggtctggttgcttctaaacagtctttcctgtggaacgttcgtccgggtttcgttaaaggttacgaatggatcgaactgctgccggacggtttcctgggtgaaaaaggtcgtatcgttaaatctgctccgcagcaggaagttctggctcacaaagctatcggtgctttctggacccacggtggttggaacggtaccatggaagctgtttgcgaaggtgttccgatgatcttctctgacttcggtctggaccagccgctgaacgctcgttacatgtctgaagttctgcacgttggtgtttacctggaaaacggtttcatccgtggtgaaatcatcaacgctgttcgtcgtgttatggttgacccggaaggtgaagttatgcgtcagaacgctcgtaaactgaaagacaaactggaccgttctatcgctccgggtggttcttcttacgaatctctggaacgtctgcagtcttacatctcttctctg

SEQ ID NO: 99 - DNA, 1371 bp, Artificial Sequence
  Enz.23
atgccgaacaccaacccgaccaccgttcgtcgtcgtcgtgttatcatgttcccggttccgttcccgggtcacctgaacccgatgctgcagctggctaacgttctgtaccgtcgtggtttcgaaatcaccatcctgcacaccaacttcaacgctccgaaaacctctctgtacccgcacttccagttccgtttcatcctggacaacgacccgcagccggaatggctgcgtaacctgccgaccaccggtccgggtgttggtgctcgtatcccggttatcaacaaacacggtgctgacgaattccgtaaagaactggaaatctgcatgcgtgacaccccgtctgacgaagaagttgcttgcgttatcaccgacgctctgtggtacttcgctcagccggttgctgactctctgaacctgaaacgtctggttctgcagaccggttctctgttcaacttccactgcctggtttgcctgccgaaattcctggaactgggttacctggacccggaaaccaaacaccgtccggacgaaccggttgttggtttcccgatgctgaaagttaaagacatccgtcgtgcttactctcacatccaggaatctaaaccgatcctgatgaaaatggttgaagaaacccgtgcttcttctggtgttatctggaactctgctaaagaactggaagaatctgaactggaaaccatccagcgtgaaatcccggctccgtctttcctgctgccgctgccgaaacactaccgtgcttcttctacctctctgctggacaccgacccgtctaccgctcagtggctggaccagcagccgccgtcttctgttctgtacgttggtttcggttctcagtcttctctggacccggctgacttcctggaaatcgctcgtggtctggttgcttctaaacagtctttcctgtggaacgttcgtccgggtttcgttaaaggttacgaatggatcgaactgctgccggacggtttcctgggtgaaaaaggtcgtatcgttaaatctgctccgcagcaggaagttctggctcacaaagctatcggtgctttctggacccacggtggttggaacggtaccatggaagctgtttgcgaaggtgttccgatgatcttctctgacttcggtctggaccagccgctgaacgctcgttacatgtctgaagttctgcacgttggtgtttacctggaaaacggtttcatccgtggtgaaatcatcaacgctgttcgtcgtgttatggttgacccggacggtgaagttatgcgtcagaacgctcgtaaactgaaagacaaactggaccgttctatcgctccgggtggttcttcttacgaatctctggaacgtctgcagtcttacatctcttctctg

SEQ ID NO: 100 - DNA, 1371 bp, Artificial Sequence
  Enz.24
atgccgaacaccaacccgaccaccgttcgtcgtcgtcgtgttatcatgttcccggttccgttcccgggtcacctgaacccgatgctgcagctggctaacgttctgtaccgtcgtggtttcgaaatcaccatcctgcacaccaacttcaacgctccgaaaacctctctgtacccgcacttccagttccgtttcatcctggacaacgacccgcagccggaatggctgcgtaacctgccgaccaccggtccgggtgttggtgctcgtatcccggttatcaacaaacacggtgctgacgaattccgtaaagaactggaaatctgcatgcgtgacaccccgtctgacgaagaagttgcttgcgttatcaccgacgctctgtggtacttcgctcagccggttgctgactctctgaacctgaaacgtctggttctgcagaccggttctctgttcaacttccactgcctggtttgcctgccgaaattcctggaactgggttacctggacccggaaaccaaacaccgtccggacgaaccggttgttggtttcccgatgctgaaagttaaagacatccgtcgtgcttactctcacatccaggaatctaaaccgatcctgatgaaaatggttgaagaaacccgtgcttcttctggtgttatctggaactctgctaaagaactggaagaatctgaactggaaaccatccagcgtgaaatcccggctccgtctttcctgctgccgctgccgaaacactaccgtgcttcttctacctctctgctggacaccgacccgtctaccgctcagtggctggaccagcagccgccgtcttctgttctgtacgttggtttcggttctcagtcttctctggacccggctgacttcctggaaatcgctcgtggtctggttgcttctaaacagtctttcctgtggaacgttcgtccgggtttcgttaaaggttacgaatggatcgaactgctgccggacggtttcctgggtgaaaaaggtcgtatcgttaaatctgctccgcagcaggaagttctggctcacaaagctatcggtgctttctggacccacggtggttggaacggtaccatggaagctgtttgcgaaggtgttccgatgatcttctctgacttcggtctggaccagccgctgaacgctcgttacatgtctgaagttctgcacgttggtgtttacctggaaaacggtttcatccgtggtgaaatcatcaacgctgttcgtcgtgttatggttgacccggaaggtgaagttatgcgtcagaacgctcgtaaactgaaagacaaactggaccgttctatcgctccgggtggttcttcttacgaatctctggaacgtctggaatcttacatctcttctctg

SEQ ID NO: 101 - DNA, 1371 bp, Artificial Sequence
  Enz.25
atgccgaacaccaacccgaccaccgttcgtcgtcgtcgtgttatcatgttcccggttccgttcccgggtcacctgaacccgatgctgcagctggctaacgttctgtaccgtcgtggtttcgaaatcaccatcctgcacaccaacttcaacgctccgaaaacctctctgtacccgcacttccagttccgtttcatcctggacaacgacccgcagccggaatggctgcgtaacctgccgaccaccggtccgggtgttggtgctcgtatcccggttatcaacaaacacggtgctgacgaattccgtaaagaactggaaatctgcatgcgtgacaccccgtctgacgaagaagttgcttgcgttatcaccgacgctctgtggtacttcgctcagccggttgctgactctctgaacctgaaacgtctggttctgcagaccggttctctgttcaacttccactgcctggtttgcctgccgaaattcctggaactgggttacctggacccggaaaccaaacaccgtccggacgaaccggttgttggtttcccgatgctgaaagttaaagacatccgtcgtgcttactctcacatccaggaatctaaaccgatcctgatgaaaatggttgaagaaacccgtgcttcttctggtgttatctggaactctgctaaagaactggaagaatctgaactggaaaccatccagcgtgaaatcccggctccgtctttcctgctgccgctgccgaaacactaccgtgcttcttctacctctctgctggacaccgacccgtctaccgctcagtggctggaccagcagccgccgtcttctgttctgtacgttggtttcggttctcagtcttctctggacccggctgacttcctggaaatcgctcgtggtctggttgcttctaaacagtctttcctgtggaacgttcgtccgggtttcgttaaaggttacgaatggatcgaactgctgccggacggtttcctgggtgaaaaaggtcgtatcgttaaatctgctccgcagcaggaagttctggctcacaaagctatcggtgctttctggacccacggtggttggaacggtaccatggaagctgtttgcgaaggtgttccgatgatcttctctgacttcggtctggaccagccgctgaacgctcgttacatgtctgaagttctgcacgttggtgtttacctggaaaacggtttcatccgtggtgaaatcatcaacgctgttcgtcgtgttatggttgacccggaaggtgaagttatgcgtcagaacgctcgtaaactgaaagacaaactggaccgttctatcgctccgggtggttcttcttacgaatctctggaacgtctgcagtcttacatccgttctctg

SEQ ID NO: 102 - DNA, 1371 bp, Artificial Sequence
  Enz.26
atgccgaacaccaacccgaccaccgttcgtcgtcgtcgtgttatcatgttcccggttccgttcccgggtcacctgaacccgatgctgcagctggctaacgttctgtaccgtcgtggtttcgaaatcaccatcctgcacaccaacttcaacgctccgaaaacctctctgtacccgcacttccagttccgtttcatcctggacaacgacccgcagccggaatggctgcgtaacctgccgaccaccggtccgggtgttggtgctcgtatcccggttatcaacaaacacggtgctgacgaattccgtaaagaactggaaatctgcatgcgtgacaccccgtctgacgaagaagttgcttgcgttatcaccgacgctctgtggtacttcgctcagccggttgctgactctctgaacctgaaacgtctggttctgcagaccggttctctgttcaacttccactgcctggtttgcctgccgaaattcctggaactgggttacctggacccggaaaccaaacaccgtccggacgaaccggttgttggtttcccgatgctgaaagttaaagacatccgtcgtgcttactctcacatccaggaatctaaaccgatcctgatgaaaatggttgaagaaacccgtgcttcttctggtgttatctggaactctgctaaagaactggaagaatctgaactggaaaccatccagcgtgaaatcccggctccgtctttcctgctgccgctgccgaaacactaccgtgcttcttctacctctctgctggacaccgacccgtctaccgctgaatggctggaccagcagccgccgtcttctgttctgtacgttggtttcggttctcagtcttctctggacccggctgacttcctggaaatcgctcgtggtctggttgcttctaaacagtctttcctgtggaacgttcgtccgggtttcgttaaaggttacgaatggatcgaactgctgccggacggtttcctgggtgaaaaaggtcgtatcgttaaatctgctccgcagcaggaagttctggctcacaaagctatcggtgctttctggacccacggtggttggaacggtaccatggaagctgtttgcgaaggtgttccgatgatcttctctgacttcggtctggaccagccgctgaacgctcgttacatgtctgaagttctgcacgttggtgtttacctggaaaacggtttcatccgtggtgaaatcatcaacgctgttcgtcgtgttatggttgacccggaaggtgaagttatgcgtcagaacgctcgtaaactgaaagacaaactggaccgttctatcgctccgggtggttcttcttacgaatctctggaacgtctgcagtcttacatctcttctctg

SEQ ID NO: 103 - DNA, 1371 bp, Artificial Sequence
  Enz.27
atgccgaacaccaacccgaccaccgttcgtcgtcgtcgtgttatcatgttcccggttccgttcccgggtcacctgaacccgatgctgcagctggctaacgttctgtaccgtcgtggtttcgaaatcaccatcctgcacaccaacttcaacgctccgaaaacctctctgtacccgcacttccagttccgtttcatcctggacaacgacccgcagccggaatggctgcgtaacctgccgaccaccggtccgggtgttggtgctcgtatcccggttatcaacaaacacggtgctgacgaattccgtaaagaactggaaatctgcatgcgtgacaccccgtctgacgaagaagttgcttgcgttatcaccgacgctctgtggtacttcgctcagccggttgctgactctctgaacctgaaacgtctggttctgcagaccggttctctgttcaacttccactgcctggtttgcctgccgaaattcctggaactgggttacctggacccggaaaccaaacaccgtccggacgaaccggttgttggtttcccgatgctgaaagttaaagacatccgtcgtgcttactctcacatccaggaatctaaaccgatcctgatgaaaatggttgaagaaacccgtgcttcttctggtgttatctggaactctgctaaagaactggaagaatctgaactggaaaccatccagcgtgaaatcccggctccgtctttcctgctgccgctgccgaaacactaccgtgcttcttctacctctctgctggacaccgacccgtctaccgctcagtggctggaccagcaggctccgtcttctgttctgtacgttggtttcggttctcagtcttctctggacccggctgacttcctggaaatcgctcgtggtctggttgcttctaaacagtctttcctgtggaacgttcgtccgggtttcgttaaaggttacgaatggatcgaactgctgccggacggtttcctgggtgaaaaaggtcgtatcgttaaatctgctccgcagcaggaagttctggctcacaaagctatcggtgctttctggacccacggtggttggaacggtaccatggaagctgtttgcgaaggtgttccgatgatcttctctgacttcggtctggaccagccgctgaacgctcgttacatgtctgaagttctgcacgttggtgtttacctggaaaacggtttcatccgtggtgaaatcatcaacgctgttcgtcgtgttatggttgacccggaaggtgaagttatgcgtcagaacgctcgtaaactgaaagacaaactggaccgttctatcgctccgggtggttcttcttacgaatctctggaacgtctgcagtcttacatctcttctctg

SEQ ID NO: 104 - DNA, 1371 bp, Artificial Sequence
  Enz.28
atgccgaacaccaacccgaccaccgttcgtcgtcgtcgtgttatcatgttcccggttccgttcccgggtcacctgaacccgatgctgcagctggctaacgttctgtaccgtcgtggtttcgaaatcaccatcctgcacaccaacttcaacgctccgaaaacctctctgtacccgcacttccagttccgtttcatcctggacaacgacccgcagccggaatggctgcgtaacctgccgaccaccggtccgggtgttggtgctcgtatcccggttatcaacaaacacggtgctgacgaattccgtaaagaactggaaatctgcatgcgtgacaccccgtctgacgaagaagttgcttgcgttatcaccgacgctctgtggtacttcgctcagccggttgctgactctctgaacctgaaacgtctggttctgcagaccggttctctgttcaacttccactgcctggtttgcctgccgaaattcctggaactgggttacctggacccggaaaccaaacaccgtccggacgaaccggttgttggtttcccgatgctgaaagttaaagacatccgtcgtgcttactctcacatccaggaatctaaaccgatcctgatgaaaatggttgaagaaacccgtgcttcttctggtgttatctggaactctgctaaagaactggaagaatctgaactggaaaccatccagcgtgaaatcccggctccgtctttcctgctgccgctgccgaaacactaccgtgcttcttctacctctctgctggacaccgacccgtctaccgctcagtggctggaccagcagccgccgtcttctgttctgtacgttggtttcggttctcagtcttctctggacccggctgacttcctggaaatcgctcgtggtctggttgcttctaaacagtctttcctgtggaacgttcgtccgggtttcgttaaaggttacgaatggatcgaactgctgccggacggtttcctgggtgaaaaaggtaaaatcgttaaatctgctccgcagcaggaagttctggctcacaaagctatcggtgctttctggacccacggtggttggaacggtaccatggaagctgtttgcgaaggtgttccgatgatcttctctgacttcggtctggaccagccgctgaacgctcgttacatgtctgaagttctgcacgttggtgtttacctggaaaacggtttcatccgtggtgaaatcatcaacgctgttcgtcgtgttatggttgacccggaaggtgaagttatgcgtcagaacgctcgtaaactgaaagacaaactggaccgttctatcgctccgggtggttcttcttacgaatctctggaacgtctgcagtcttacatctcttctctg

SEQ ID NO: 105 - DNA, 1371 bp, Artificial Sequence
  Enz.29
atgccgaacaccaacccgaccaccgttcgtcgtcgtcgtgttatcatgttcccggttccgttcccgggtcacctgaacccgatgctgcagctggctaacgttctgtaccgtcgtggtttcgaaatcaccatcctgcacaccaacttcaacgctccgaaaacctctctgtacccgcacttccagttccgtttcatcctggacaacgacccgcagccggaatggctgcgtaacctgccgaccaccggtccgggtgttggtgctcgtatcccggttatcaacaaacacggtgctgacgaattccgtaaagaactggaaatctgcatgcgtgacaccccgtctgacgaagaagttgcttgcgttatcaccgacgctctgtggtacttcgctcagccggttgctgactctctgaacctgaaacgtctggttctgcagaccggttctctgttcaacttccactgcctggtttgcctgccgaaattcctggaactgggttacctggacccggaaaccaaacaccgtccggacgaaccggttgttggtttcccgatgctgaaagttaaagacatccgtcgtgcttactctcacatccaggaatctaaaccgatcctgatgaaaatggttgaagaaacccgtgcttcttctggtgttatctggaactctgctaaagaactggaagaatctgaactggaaaccatccagcgtgaaatcccggctccgtctttcctgctgccgctgccgaaacactaccgtgcttcttctacctctctgctggacaccgacccgtctaccgctcagtggctggaccagcagccgccgtcttctgttctgtacgttggtttcggttctcagtcttctctggacccggctgacttcctggaaatcgctcgtggtctggttgcttctaaacagtctttcctgtggaacgttcgtccgggtttcgttaaaggttacgaatggatcgaactgctgccggacggtttcctgggtgaaaaaggtcgtatcgttaaatctgctccgcagcaggaagttctggctcacccggctatcggtgctttctggacccacggtggttggaacggtaccatggaagctgtttgcgaaggtgttccgatgatcttctctgacttcggtctggaccagccgctgaacgctcgttacatgtctgaagttctgcacgttggtgtttacctggaaaacggtttcatccgtggtgaaatcatcaacgctgttcgtcgtgttatggttgacccggaaggtgaagttatgcgtcagaacgctcgtaaactgaaagacaaactggaccgttctatcgctccgggtggttcttcttacgaatctctggaacgtctgcagtcttacatctcttctctg

SEQ ID NO: 106 - DNA, 1371 bp, Artificial Sequence
  Enz.30
atgccgaacaccaacccgaccaccgttcgtcgtcgtcgtgttatcatgttcccggttccgttcccgggtcacctgaacccgatgctgcagctggctaacgttctgtaccgtcgtggtttcgaaatcaccatcctgcacaccaacttcaacgctccgaaaacctctctgtacccgcacttccagttccgtttcatcctggacaacgacccgcagccggaatggctgcgtaacctgccgaccaccggtccgggtgttggtgctcgtatcccggttatcaacaaacacggtgctgacgaattccgtaaagaactggaaatctgcatgcgtgacaccccgtctgacgaagaagttgcttgcgttatcaccgacgctctgtggtacttcgctcagccggttgctgactctctgaacctgaaacgtctggttctgcagaccggttctctgttcaacttccactgcctggtttgcctgccgaaattcctggaactgggttacctggacccggaaaccaaacaccgtccggacgaaccggttgttggtttcccgatgctgaaagttaaagacatccgtcgtgcttactctcacatccaggaatctaaaccgatcctgatgaaaatggttgaagaaacccgtgcttcttctggtgttatctggaactctgctaaagaactggaagaatctgaactggaaaccatccagcgtgaaatcccggctccgtctttcctgctgccgctgccgaaacactaccgtgcttcttctacctctctgctggacaccgacccgtctaccgctcagtggctggaccagcagccgccgtcttctgttctgtacgttggtttcggttctcagtcttctctggacccggctgacttcctggaaatcgctcgtggtctggttgcttctaaacagtctttcctgtggaacgttcgtccgggtttcgttaaaggttacgaatggatcgaactgctgccggacggtttcctgggtgaaaaaggtcgtatcgttaaatctgctccgcagcaggaagttctggctcacaaagctatcggtgctttctggacccacggtggttggaacggtaccatggaagctgtttgcgaaggtgttccgatgatcttctctgacttcggtggtgaccagccgctgaacgctcgttacatgtctgaagttctgcacgttggtgtttacctggaaaacggtttcatccgtggtgaaatcatcaacgctgttcgtcgtgttatggttgacccggaaggtgaagttatgcgtcagaacgctcgtaaactgaaagacaaactggaccgttctatcgctccgggtggttcttcttacgaatctctggaacgtctgcagtcttacatctcttctctg

SEQ ID NO: 107 - DNA, 1371 bp, Artificial Sequence
  Enz.31
atgccgaacaccaacccgaccaccgttcgtcgtcgtcgtgttatcatgttcccggttccgttcccgggtcacctgaacccgatgctgcagctggctaacgttctgtaccgtcgtggtttcgaaatcaccatcctgcacaccaacttcaacgctccgaaaacctctctgtacccgcacttccagttccgtttcatcctggacaacgacccgcagccggaatggctgcgtaacctgccgaccaccggtccgggtgttggtgctcgtatcccggttatcaacaaacacggtgctgacgaattccgtaaagaactggaaatctgcatgcgtgacaccccgtctgacgaagaagttgcttgcgttatcaccgacgctctgtggtacttcgctcagccggttgctgactctctgaacctgaaacgtctggttctgcagaccggttctctgttcaacttccactgcctggtttgcctgccgaaattcctggaactgggttacctggacccggaaaccaaacaccgtccggacgaaccggttgttggtttcccgatgctgaaagttaaagacatccgtcgtgcttactctcacatccaggaatctaaaccgatcctgatgaaaatggttgaagaaacccgtgcttcttctggtgttatctggaactctgctaaagaactggaagaatctgaactggaaaccatccagcgtgaaatcccggctccgtctttcctgctgccgctgccgaaacactaccgtgcttcttctacctctctgctggacaccgacccgtctaccgctgaatggctggaccagcaggctccgtcttctgttctgtacgttggtttcggttctcagtcttctctggacccggctgacttcctggaaatcgctcgtggtctggttgcttctaaacagtctttcctgtggaacgttcgtccgggtttcgttaaaggttacgaatggatcgaactgctgccggacggtttcctgggtgaaaaaggtcgtatcgttaaatctgctccgcagcaggaagttctggctcacaaagctatcggtgctttctggacccacggtggttggaacggtaccatggaagctgtttgcgaaggtgttccgatgatcttctctgacttcggtctggaccagccgctgaacgctcgttacatgtctgaagttctgcacgttggtgtttacctggaaaacggtttcatccgtggtgaaatcatcaacgctgttcgtcgtgttatggttgacccggaaggtgaagttatgcgtcagaacgctcgtaaactgaaagacaaactggaccgttctatcgctccgggtggttcttcttacgaatctctggaacgtctgcagtcttacatctcttctctg

SEQ ID NO: 108 - DNA, 1371 bp, Artificial Sequence
  Enz.32
atgccgaacaccaacccgaccaccgttcgtcgtcgtcgtgttatcatgttcccggttccgttcccgggtcacctgaacccgatgctgcagctggctaacgttctgtaccgtcgtggtttcgaaatcaccatcctgcacaccaacttcaacgctccgaaaacctctctgtacccgcacttccagttccgtttcatcctggacaacgacccgcagccggaatggctgcgtaacctgccgaccaccggtccgggtgttggtgctcgtatcccggttatcaacaaacacggtgctgacgaattccgtaaagaactggaaatctgcatgcgtgacaccccgtctgacgaagaagttgcttgcgttatcaccgacgctctgtggtacttcgctcagccggttgctgactctctgaacctgaaacgtctggttctgcagaccggttctctgttcaacttccactgcctggtttgcctgccgaaattcctggaactgggttacctggacccggaaaccaaacaccgtccggacgaaccggttgttggtttcccgatgctgaaagttaaagacatccgtcgtgcttactctcacatccaggaatctaaaccgatcctgatgaaaatggttgaagaaacccgtgcttcttctggtgttatctggaactctgctaaagaactggaagaatctgaactggaaaccatccagcgtgaaatcccggctccgtctttcctgctgccgctgccgaaacactaccgtgcttcttctacctctctgctggacaccgacccgtctaccgctcagtggctggaccagcagccgccgtcttctgttctgtacgttggtttcggttctcagtcttctctggacccggctgacttcctggaaatcgctcgtggtctggttgcttctaaacagtctttcctgtggaacgttcgtccgggtttcgttaaaggttacgaatggatcgaactgctgccggacggtttcctgggtgaaaaaggtaaaatcgttaaatctgctccgcagcaggaagttctggctcacccggctatcggtgctttctggacccacggtggttggaacggtaccatggaagctgtttgcgaaggtgttccgatgatcttctctgacttcggtctggaccagccgctgaacgctcgttacatgtctgaagttctgcacgttggtgtttacctggaaaacggtttcatccgtggtgaaatcatcaacgctgttcgtcgtgttatggttgacccggaaggtgaagttatgcgtcagaacgctcgtaaactgaaagacaaactggaccgttctatcgctccgggtggttcttcttacgaatctctggaacgtctgcagtcttacatctcttctctg

SEQ ID NO: 109 - DNA, 1371 bp, Artificial Sequence
  Enz.33
atgccgaacaccaacccgaccaccgttcgtcgtcgtcgtgttatcatgttcccggttccgttcccgggtcacctgaacccgatgctgcagctggctaacgttctgtaccgtcgtggtttcgaaatcaccatcctgcacaccaacttcaacgctccgaaaacctctctgtacccgcacttccagttccgtttcatcctggacaacgacccgcagccggaatggctgcgtaacctgccgaccaccggtccgggtgttggtgctcgtatcccggttatcaacaaacacggtgctgacgaattccgtaaagaactggaaatctgcatgcgtgacaccccgtctgacgaagaagttgcttgcgttatcaccgacgctctgtggtacttcgctcagccggttgctgactctctgaacctgaaacgtctggttctgcagaccggttctctgttcaacttccactgcctggtttgcctgccgaaattcctggaactgggttacctggacccggaaaccaaacaccgtccggacgaaccggttgttggtttcccgatgctgaaagttaaagacatccgtcgtgcttactctcacatccaggaatctaaaccgatcctgatgaaaatggttgaagaaacccgtgcttcttctggtgttatctggaactctgctaaagaactggaagaatctgaactggaaaccatccagcgtgaaatcccggctccgtctttcctgctgccgctgccgaaacactaccgtgcttcttctacctctctgctggacaccgacccgtctaccgctgaatggctggaccagcaggctccgtcttctgttctgtacgttggtttcggttctcagtcttctctggacccggctgacttcctggaaatcgctcgtggtctggttgcttctaaacagtctttcctgtggaacgttcgtccgggtttcgttaaaggttacgaatggatcgaactgctgccggacggtttcctgggtgaaaaaggtcgtatcgttaaatctgctccgcagcaggaagttctggctcacaaagctatcggtgctttctggacccacggtggttggaacggtaccatggaagctgtttgcgaaggtgttccgatgatcttctctgacttcggtggtgaccagccgctgaacgctcgttacatgtctgaagttctgcacgttggtgtttacctggaaaacggtttcatccgtggtgaaatcatcaacgctgttcgtcgtgttatggttgacccggaaggtgaagttatgcgtcagaacgctcgtaaactgaaagacaaactggaccgttctatcgctccgggtggttcttcttacgaatctctggaacgtctgcagtcttacatctcttctctg

SEQ ID NO: 110 - DNA, 1371 bp, Artificial Sequence
  Enz.34
atgccgaacaccaacccgaccaccgttcgtcgtcgtcgtgttatcatgttcccggttccgttcccgggtcacctgaacccgatgctgcagctggctaacgttctgtaccgtcgtggtttcgaaatcaccatcctgcacaccaacttcaacgctccgaaaacctctctgtacccgcacttccagttccgtttcatcctggacaacgacccgcagccggaatggctgcgtaacctgccgaccaccggtccgggtgttggtgctcgtatcccggttatcaacaaacacggtgctgacgaattccgtaaagaactggaaatctgcatgcgtgacaccccgtctgacgaagaagttgcttgcgttatcaccgacgctctgtggtacttcgctcagccggttgctgactctctgaacctgaaacgtctggttctgcagaccggttctctgttcaacttccactgcctggtttgcctgccgaaattcctggaactgggttacctggacccggaaaccaaacaccgtccggacgaaccggttgttggtttcccgatgctgaaagttaaagacatccgtcgtgcttactctcacatccaggaatctaaaccgatcctgatgaaaatggttgaagaaacccgtgcttcttctggtgttatctggaactctgctaaagaactggaagaatctgaactggaaaccatccagcgtgaaatcccggctccgtctttcctgctgccgctgccgaaacactaccgtgcttcttctacctctctgctggacaccgacccgtctaccgctgaatggctggaccagcaggctccgtcttctgttctgtacgttggtttcggttctcagtcttctctggacccggctgacttcctggaaatcgctcgtggtctggttgcttctaaacagtctttcctgtggaacgttcgtccgggtttcgttaaaggttacgaatggatcgaactgctgccggacggtttcctgggtgaaaaaggtaaaatcgttaaatctgctccgcagcaggaagttctggctcacccggctatcggtgctttctggacccacggtggttggaacggtaccatggaagctgtttgcgaaggtgttccgatgatcttctctgacttcggtctggaccagccgctgaacgctcgttacatgtctgaagttctgcacgttggtgtttacctggaaaacggtttcatccgtggtgaaatcatcaacgctgttcgtcgtgttatggttgacccggaaggtgaagttatgcgtcagaacgctcgtaaactgaaagacaaactggaccgttctatcgctccgggtggttcttcttacgaatctctggaacgtctgcagtcttacatctcttctctg

SEQ ID NO: 111 - DNA, 1371 bp, Artificial Sequence
  Enz.35
atgccgaacaccaacccgaccaccgttcgtcgtcgtcgtgttatcatgttcccggttccgttcccgggtcacctgaacccgatgctgcagctggctaacgttctgtaccgtcgtggtttcgaaatcaccatcctgcacaccaacttcaacgctccgaaaacctctctgtacccgcacttccagttccgtttcatcctggacaacgacccgcagccggaatggctgcgtaacctgccgaccaccggtccgggtgttggtgctcgtatcccggttatcaacaaacacggtgctgacgaattccgtaaagaactggaaatctgcatgcgtgacaccccgtctgacgaagaagttgcttgcgttatcaccgacgctctgtggtacttcgctcagccggttgctgactctctgaacctgaaacgtctggttctgcagaccggttctctgttcaacttccactgcctggtttgcctgccgaaattcctggaactgggttacctggacccggaaaccaaacaccgtccggacgaaccggttgttggtttcccgatgctgaaagttaaagacatccgtcgtgcttactctcacatccaggaatctaaaccgatcctgatgaaaatggttgaagaaacccgtgcttcttctggtgttatctggaactctgctaaagaactggaagaatctgaactggaaaccatccagcgtgaaatcccggctccgtctttcctgctgccgctgccgaaacactaccgtgcttcttctacctctctgctggacaccgacccgtctaccgctgaatggctggaccagcaggctccgtcttctgttctgtacgttggtttcggttctcagtcttctctggacccggctgacttcctggaaatcgctcgtggtctggttgcttctaaacagtctttcctgtggaacgttcgtccgggtttcgttaaaggttacgaatggatcgaactgctgccggacggtttcctgggtgaaaaaggtaaaatcgttaaatctgctccgcagcaggaagttctggctcacccggctatcggtgctttctggacccacggtggttggaacggtaccatggaagctgtttgcgaaggtgttccgatgatcttctctgacttcggtggtgaccagccgctgaacgctcgttacatgtctgaagttctgcacgttggtgtttacctggaaaacggtttcatccgtggtgaaatcatcaacgctgttcgtcgtgttatggttgacccggaaggtgaagttatgcgtcagaacgctcgtaaactgaaagacaaactggaccgttctatcgctccgggtggttcttcttacgaatctctggaacgtctgcagtcttacatctcttctctg

SEQ ID NO: 112 - protein, 457 aa, Artificial Sequence
  Enz.11µÄ°±»ùËáÐòÁÐ
MPNTNPTTVRRRRVIMFPVPFPGHLNPMLQLANVLYRRGFEITILHTNFNAPKTSLYPHFQFRFILDNDPQPEWLRNLPTTGPGVGARIPVINKHGADEFRKELEICMRDTPSDEEVACVITDALWYFAQPVADSLNLKRLVLQTGSLFNFHCLVCLPKFLELGYLDPETKHRPDEPVVGFPMLKVKDIRRAYSHIQESKPILMKMVEETRASSGVIWNSAKELEESELETIQREIPAPSFLLPLPKHYRASSTSLLDTDPSTAQWLDQQPPSSVLYVGFGSQSSLDPADFLEIARGLVASKQSFLWNVRPGFVKGYEWIELLPDGFLGEKGRIVKSAPQQEVLAHKAIGAFWTHGGWNGTMEAVCEGVPMIFSDFGLDQPLNARYMSEVLHVGVYLENGFIRGEIINAVRRVMVDPEGEVMRQNARKLKDKLDRSIAPGGSSYESLERLQSYISSL